European Patent Specification EP 3 766 987 B1, published August 2, 2023. Title: ALPHA-HEMOLYSIN VARIANTS. Applicant: F. Hoffmann-La Roche AG       Roche Diagnostics GmbH. The sequence listing filed with the application follows.

SEQUENCE LISTING (11 sequences)

SEQ ID NO: 1 - DNA, 1023 bp, Staphylococcus aureus
atggcagatctcgatcccgcgaaattaatacgactcactatagggaggccacaacggtttccctctagaaataattttgtttaactttaagaaggagatatacaaatggattcagatattaatattaaaacaggtacaacagatattggttcaaatacaacagtaaaaactggtgatttagtaacttatgataaagaaaatggtatgcataaaaaagtattttattcttttattgatgataaaaatcataataaaaaattgttagttattcgtacaaaaggtactattgcaggtcaatatagagtatatagtgaagaaggtgctaataaaagtggtttagcatggccatctgcttttaaagttcaattacaattacctgataatgaagtagcacaaatttcagattattatccacgtaatagtattgatacaaaagaatatatgtcaacattaacttatggttttaatggtaatgtaacaggtgatgatactggtaaaattggtggtttaattggtgctaatgtttcaattggtcatacattaaaatatgtacaaccagattttaaaacaattttagaaagtcctactgataaaaaagttggttggaaagtaatttttaataatatggttaatcaaaattggggtccttatgatcgtgatagttggaatcctgtatatggtaatcaattatttatgaaaacaagaaatggttctatgaaagcagctgataatttcttagatccaaataaagcatcaagtttattatcttcaggtttttctcctgattttgcaacagttattactatggatagaaaagcatcaaaacaacaaacaaatattgatgttatttatgaacgtgtaagagatgattatcaattacattggacatcaactaattggaaaggtacaaatactaaagataaatggacagatagaagttcagaaagatataaaattgattgggaaaaagaagaaatgacaaatggtctcagcgcttggagccacccgcagttcgaaaaataa

SEQ ID NO: 2 - protein, 306 aa, Staphylococcus aureus
MADSDINIKTGTTDIGSNTTVKTGDLVTYDKENGMHKKVFYSFIDDKNHNKKLLVIRTKGTIAGQYRVYSEEGANKSGLAWPSAFKVQLQLPDNEVAQISDYYPRNSIDTKEYMSTLTYGFNGNVTGDDTGKIGGLIGANVSIGHTLKYVQPDFKTILESPTDKKVGWKVIFNNMVNQNWGPYDRDSWNPVYGNQLFMKTRNGSMKAADNFLDPNKASSLLSSGFSPDFATVITMDRKASKQQTNIDVIYERVRDDYQLHWTSTNWKGTNTKDKWTDRSSERYKIDWEKEEMTNGLSAWSHPQFEK

SEQ ID NO: 3 - protein, 305 aa, Staphylococcus aureus
ADSDINIKTGTTDIGSNTTVKTGDLVTYDKENGMHKKVFYSFIDDKNHNKKLLVIRTKGTIAGQYRVYSEEGANKSGLAWPSAFKVQLQLPDNEVAQISDYYPRNSIDTKEYMSTLTYGFNGNVTGDDTGKIGGLIGANVSIGHTLKYVQPDFKTILESPTDKKVGWKVIFNNMVNQNWGPYDRDSWNPVYGNQLFMKTRNGSMKAADNFLDPNKASSLLSSGFSPDFATVITMDRKASKQQTNIDVIYERVRDDYQLHWTSTNWKGTNTKDKWTDRSSERYKIDWEKEEMTNGLSAWSHPQFEK

SEQ ID NO: 4 - protein, 305 aa, Artificial Sequence
  source: /note="Description of Artificial Sequence: Synthetic polypeptide"
ADSDINIKTGTTDIGSKTTVKTGDLVTYDKENGMHKKVFYSFIDDKNHNKKLLVIRTKGTIAGQYRVYSEEGANKSGLAWPSAFKVQLQLPDNEVAQISDYYPRNSIDTKEYMSTLTYGFNGNVTGDDTGKIGGLIGANVSIGHTLKYVQPDFKTILESPTDKKVGWKVIFNNMVNQNWGPYDRDSWNPVYGNQLFMKTRNGSMKAADNFLDPNKASSLLSSGFSPDFATVITMDRKASKQQTNIDVIYERVRDDYQLHWTSTNWKGTNTKDKWTDRSSERYKIDWEKEEMTNGLSAWSHPQFEK

SEQ ID NO: 5 - protein, 305 aa, Artificial Sequence
  source: /note="Description of Artificial Sequence: Synthetic polypeptide"
ADSDINIKTGTTDIGSRTTVKTGDLVTYDKENGMHKKVFYSFIDDKNHNKKLLVIRTKGTIAGQYRVYSEEGANKSGLAWPSAFKVQLQLPDNEVAQISDYYPRNSIDTKEYMSTLTYGFNGNVTGDDTGKIGGLIGANVSIGHTLKYVQPDFKTILESPTDKKVGWKVIFNNMVNQNWGPYDRDSWNPVYGNQLFMKTRNGSMKAADNFLDPNKASSLLSSGFSPDFATVITMDRKASKQQTNIDVIYERVRDDYQLHWTSTNWKGTNTKDKWTDRSSERYKIDWEKEEMTNGLSAWSHPQFEK

SEQ ID NO: 6 - protein, 305 aa, Artificial Sequence
  source: /note="Description of Artificial Sequence: Synthetic polypeptide"
ADSDINIKTGTKDIGSNTTVKTGDLVTYDKENGMHKKVFYSFIDDKNHNKKLLVIRTKGTIAGQYRVYSEEGANKSGLAWPSAFKVQLQLPDNEVAQISDYYPRNSIDTKEYMSTLTYGFNGNVTGDDTGKIGGLIGANVSIGHTLKYVQPDFKTILESPTDKKVGWKVIFNNMVNQNWGPYDRDSWNPVYGNQLFMKTRNGSMKAADNFLDPNKASSLLSSGFSPDFATVITMDRKASKQQTNIDVIYERVRDDYQLHWTSTNWKGTNTKDKWTDRSSERYKIDWEKEEMTNGLSAWSHPQFEK

SEQ ID NO: 7 - protein, 305 aa, Artificial Sequence
  source: /note="Description of Artificial Sequence: Synthetic polypeptide"
ADSDINIKTGTRDIGSNTTVKTGDLVTYDKENGMHKKVFYSFIDDKNHNKKLLVIRTKGTIAGQYRVYSEEGANKSGLAWPSAFKVQLQLPDNEVAQISDYYPRNSIDTKEYMSTLTYGFNGNVTGDDTGKIGGLIGANVSIGHTLKYVQPDFKTILESPTDKKVGWKVIFNNMVNQNWGPYDRDSWNPVYGNQLFMKTRNGSMKAADNFLDPNKASSLLSSGFSPDFATVITMDRKASKQQTNIDVIYERVRDDYQLHWTSTNWKGTNTKDKWTDRSSERYKIDWEKEEMTNGLSAWSHPQFEK

SEQ ID NO: 8 - protein, 293 aa, Staphylococcus aureus
ADSDINIKTGTTDIGSNTTVKTGDLVTYDKENGMHKKVFYSFIDDKNHNKKLLVIRTKGTIAGQYRVYSEEGANKSGLAWPSAFKVQLQLPDNEVAQISDYYPRNSIDTKEYMSTLTYGFNGNVTGDDTGKIGGLIGANVSIGHTLKYVQPDFKTILESPTDKKVGWKVIFNNMVNQNWGPYDRDSWNPVYGNQLFMKTRNGSMKAADNFLDPNKASSLLSSGFSPDFATVITMDRKASKQQTNIDVIYERVRDDYQLHWTSTNWKGTNTKDKWTDRSSERYKIDWEKEEMTN

SEQ ID NO: 9 - protein, 10 aa, Artificial Sequence
  source: /note="Description of Artificial Sequence: Synthetic peptide"
GSGSGSGSGS

SEQ ID NO: 10 - protein, 6 aa, Artificial Sequence
  source: /note="Description of Artificial Sequence: Synthetic 6xHis tag"
HHHHHH

SEQ ID NO: 11 - protein, 10 aa, Artificial Sequence
  source: /note="Description of Artificial Sequence: Synthetic peptide"
HHHHHHGSGG